European Patent Specification EP 3 950 949 B1, published December 4, 2024. Title: An immunodeficient rodent. Applicant: Central Institute for Experimental animals. The sequence listing filed with the application follows.

SEQUENCE LISTING (2 sequences)

SEQ ID NO: 1 - DNA, 3653 bp, Homo sapiens
atgagtcatggggggcgggggggtttctgggggagttcccagctaatcaacttgggacaggacagcctggaactttcgatggtgcctatccaagtgtggggtgggcacagcagccaagacccaatgtccttatctcaggtaggggctcaggaggtctcccagacaggcagcctccggagagtttgggggtaggaatgggagcaaccagcttctttttttctctcttagaatttgggggcttgggggacaggcttgagaatcccaaaggagaggggcaaaggacactgcccccgcaagtctgccagagcagagagggagaccccgactcagctgccacttccccacaggctgctgccgcttccaggcgtctatcagcggctcagcctttgttcagctgttctgttcaaacactctggggccattcaggcctgggtggggcagcgggaggaagggagtttgaggggggcaaggcgacgtcaaaggaggatcagagattccacaatttcacaaaactttcgcaaacagctttttgttccaacccccctgcattgtcttggacaccaaatttgcataaatcctgggaagttattactaagccttagtcgtggccccaggtaatttcctcccaggcctccatggggttatgtataaaggcccccctagagctgggccccaaaacagcccggagcctgcagcccagccccacccagacccatggctggacctgccacccagagccccatgaagctgatgggtgagtgtcttggcccaggatgggagagccgcctgccctggcatgggagggaggctggtgtgacagaggggctggggatccccgttctgggaatggggattaaaggcacccagtgtccccgagagggcctcaggtggtagggaacagcatgtctcctgagcccgctctgtccccagccctgcagctgctgctgtggcacagtgcactctggacagtgcaggaagccacccccctgggccctgccagctccctgccccagagcttcctgctcaagtgcttagagcaagtgaggaagatccagggcgatggcgcagcgctccaggagaagctggtgagtgaggtgggtgagagggctgtggagggaagcccggtggggagagctaagggggatggaactgcagggccaacatcctctggaagggacgtgggagaatattaggagcagtggagctggggaaggctgggaagggacttggggaggaggaccttggtggggacagtgctcgggagggctggctgggatgggagtggaggcattacattcaggagaaagggcaagggcccctgtgagatcagagagtgggggtgcagggcagagaggaactgaacagcctggcaggacatggagggaggggaaagaccagagagtcggggaggacccgggaaggagcggcgacccggccatggcgagtctcactcagcatccttccatccccagtgtgccacctacaagctgtgccaccccgaggagctggtgctgctcggacactctctgggcatcccctgggctcccctgagcagctgccccagccaggccctgcagctggtgagtgtcaggaaaggataaggctaatgaggagggggaaggagaggaggaacacccatgggctcccccatgtctccaggttccaagctgggggcctgacgtatctcaggcagcaccccctaactcttccgctctgtctcacaggcaggctgcttgagccaactccatagcggccttttcctctaccaggggctcctgcaggccctggaagggatctcccccgagttgggtcccaccttggacacactgcagctggacgtcgccgactttgccaccaccatctggcagcaggtgagccttgttgggcagggtggccaaggtcgtgctggcattctgggcaccacagccaggcctgtgtatgggccctgtccatgctgtcacccccagcatttcctcatttgtaataacgcccactcagaagggcccaaccactgatcacagctttcccccacagatggaagaactgggaatggcccctgccctgcagcccacccagggtgccatgccggccttcgcctctgctttccagcgccgggcaggaggggtcctggttgcctcccatctgcagagcttcctggaggtgtcgtaccgcgttctacgccaccttgcccagccctgagccaagccctccccatcccatgtatttatctctatttaatatttatgtctatttaagcctcatatttaaagacagggaagagcagaacggagccccaggcctctgtgtccttccctgcatttctgagtttcattctcctgcctgtagcagtgagaaaaagctcctgtcctcccatcccctggactgggaggtagataggtaaataccaagtatttattactatgactgctccccagccctggctctgcaatgggcactgggatgagccgctgtgagcccctggtcctgagggtccccacctgggacccttgagagtatcaggtctcccacgtgggagacaagaaatccctgtttaatatttaaacagcagtgttccccatctgggtccttgcacccctcactctggcctcagccgactgcacagcggcccctgcatccccttggctgtgaggcccctggacaagcagaggtggccagagctgggaggcatggccctggggtcccacgaatttgctggggaatctcgtttttcttcttaagacttttgggacatggtttgactcccgaacatcaccgacgcgtctcctgtttttctgggtggcctcgggacacctgccctgcccccacgagggtcaggactgtgactctttttagggccaggcaggtgcctggacatttgccttgctggacggggactggggatgtgggagggagcagacaggaggaatcatgtcaggcctgtgtgtgaaaggaagctccactgtcaccctccacctcttcaccccccactcaccagtgtcccctccactgtcacattgtaactgaacttcaggataataaagtgtttgcctccagtcacgtccttcctccttcttgagtccagctggtgcctggccaggggctggggaggtggctgaagggtgggagaggccagagggaggtcggggaggaggtctggggaggaggtccagggaggaggaggaaagttctcaagttcgtctgacattcattccgttagcacatatttatctgagcacctactctgtgcagacgctgggctaagtgctggggacacagcagggaacaaggcagacatggaatctgcactcgagcagccaaagcctggcagggaagacagaggcacagggaccatgggaacccggaaaggagagggcatggggtctgggtgggcttaacaggccagacacagccagacaagatgaagccagggagtgctgagcatctgcaccaggcttgtcatttaccatcttccataaacttgagcccatccatcaagttgcccacaaagtggaagccaagttcaaggtgaccactggggtcagagcttctctcctcagactcggtctctgcactcgccccagctggtcacttcctgcttgtggcagccttgggctgaagagcgctaagctcacagcccaggagggtggggagct

SEQ ID NO: 2 - DNA, 21091 bp, Mus musculus
actaggaaggttgagaaccgctgctctagagaaccctgactaatataccaatatatactattttgatgattttcaaacttagaacaatttttcccctctcttttgtgatagatgaacttacagggtgggccttttgaaaggggttacaacctgagaagataaaaccaggaacccctaggattgtacaaagcggtgagggcagggaccatggactagggaggccaggggtgggagggtctattgagagtcctggaaaatggcaggttttcagctaacaagggaagaaaacctgaagtaaacgttacctgtcctggaatcttgattcttcccgggcagaggcttcagccagactcagtgagaagagagtctcctccaccccagccctcattaattttccacgctattttgtcctgcttcgttttgaaataaacacttgaagaccccagccctcccttggccctgtcttgtctcgggtgctctgctgagcctcaaagcgaggagctcaggaaatccggagagaagggagggtggccacgggccaggttgctacaatgcccagccctctaagacccctgaggcaggaaggtccctagctcaccagtttccctcaacctccttcctgagaggaaggggctgtctatgtcccccaccccaagggtgaaggctcagccaaacgcagcagggaagccaggaaggtgtcgcaattctgggtcccccccaccccccgcctgtcattaacgacggggctagaaagagaagtttcgggaacttgccccaagaggagaggagacgagagagaagagagagcacaagcgtgggggctgggcacagcgccctagccccagtgtaagtagggggagggcggggagccctggagacctcagaccattccccaaccctgctagggccacatcagggggcccaagacaggatccttggggaaatgggagtctctctgtgtgtatagcatcagggaggtcagacagctggatctctgggaacaggagctgagctcaggtatgaagaatcccacccagagtccctatccttcagacaggcttactccctgctttcagccatttggcctgcttcttctcagcaagaacagctgtctcagagtctctgggcctctgtttcctctcccggttcccttagcctcttaactttaaacagttgatgcaagacttgcctgagatagctttctctgtcggcctctccacttctctctgcatcgctccagcctgctcatcgttgttgttgatgatgatgttgtatgcagctctcatgcagacaaggtttatcatcttgtcggcagataagaaccttgaacttcttctgatcctcctgtatcacaaatgctggtctgtaggcctccaccaccatgcctgatacttaatgtggtactggggatcaagccttggtctttgtgcctgctagacaagtgttcaaccaactaagctctatccccagccctggttgctttatatttttgagataggtttcgctaagttgccaaaatgagatttgaatgtcttctatagcacaggctggccttgatcttgtaacacacttgcccccacttccagaataactggtctcaaccccctgccactgggctaggctctacctctgtctattctctatgtatctcttttccccagcttgtctattcacccatctatgatgcattgatcctttatctctgccacacctggggatctcgctcccatagtttattctcaacatcctcttcgtccccgtcttcccacagacagaatttcaaaagaataggacaggagaagggagcccagagggaaggttggcaacaatgagcaaaaggaaaaggtagagaggatgctgtagcagcctgacttacggcatcagctgtgtccgtgggcacagtggacacagcgagcagctgcagagcccagcacatggccagagtggtgggaagagcctgagaggcttggagctagaagtagacctggtggctatgccaggaggctattggttcctttggctgatttcctgcttttagggctcatacagatagcccactgcttctgagagcttgttccttgggcactgtgccaagagctttcatcttaactgtctcgcttcatcgttatagcattgctgagacatgagtggtattgttaagcccctttttcctaaatggagaaactgagactcagaatggtgaagtaactcatccaagttcaccaggcaggtgagtgttggaaccagagtcagaactgggctcccagcctctttgtacacttcttccctagacaatgagacataggctccagcaggcccaagctcctactcaactggggccaccctcaaggcttccataggaaactgttctgatgttaaacatgccagccccatgcaatctagagaggaggcctggtctcctctgttctgttttctgctcttgacataagcctgtgggaaggatacagtggtaccaggtatgaactaggcctactacaaccacaaatgagtggagaaccagcatcctgagccctgggggctaagtctttcccactcagtgtgtacatatgtacatgtgtgtgtgcatgtggatgcaggagatgatcaaactggtatgttgatgtgaggttattgtctgaggtttccattgctaggatagaacaccctagccaaaagcaacttggaaaaagggttatttcaccatacacttccaggcaacagtccatcactgaagaaagtcagggcaggaatttgagacagaaactaatgcagatgccattgaagagtgctgctactggcttggtccccatggtttgcttagcctaacttcttgtagcactgggaccacccgtccagggatgacactacccacaatgatctggcccctcccacatccagcattcatcaggaaaatgtacctaccacaggcttgcccacaagcaaatctggtagaggtattttctcaactgaagtttcctcttcccaaatgatgctagcttgtattacgttgacacacaactagccagcacagttacaaaacaaagattggtaaacagagatatggggggggggcgcaagagggaagaaaagcttgcgccccctcctagctccatcctatccctgctctttctaggagacagatttgaccttggcagtgtgttgcacacatggacatttccttgataccctggtgaggggaaagccattgatttgaaccatttcatgtctttctcttaaaggcagtacaggccagtgtcaccccatgttgcaagcactgagactcaggggtcaggtatcctgcccagatactggcagagcaaggctctggctgcaaatcctgttcttaaccatctctcactgcctccaggtaagcttcaagctggcaaaatggtagggctgggagcctgcaccctgactggagttaccctgatcttcttgctactccccagaagtaagtcaggggccggggaggacaattataagggaggcatcggtccccccaagctgctgtgtgccagaccctgggagtgtggcagtgaacacagcagccaaagcctctccatcacagagcttcgaggtagcagagcagttatgactctcattacaaagggatgtcagaaatccaggaaacagtctggttcactgggatgcccatatgctaagctggtgagagagggcctaaagggcaccatgaagaggaggcagcagggcgaagagccacagatgggagagaagcatattgtttctccaggaatagactaggtgtctgcaagcagaaaccatggtcagagctgaaacagtgagtgaggccaggagctacacgaggggtctggaactctatcctaaccttggctgcctgtactgacccgacagctactgttcttcacaattgtgttagaatgtctgattcttttagccaggtggaggtggggcaagcctttagtcccaacatttgggaagcaaaggcagacggatctctatgagttctaggctagcctgacctacaaagtgtgttctaggacagccaaagagtcaaagagaaaacctgtcttaaataaatgaaacaaaataaaaaaaataaataaggaaaaggagcctgatgctgactcgccatagacaagcaccgagaattattatcagcagtcagggccttgataatgccagccacctagccaggggaggctggaatatggcggagatgtgacaacagcccacagaactgaggaagttccttagggggggggggtgtctgggtttagcagattagtggtagttctggctaggagataaggctaaaagtaggaagctaacctactatcctgccctatattagggcctcctgttacatgttaggatccttgcagctttgtggaggtactaggtaggattaaggcatgactggaccatcccacagggactttgggatctaactggtaggaactgttttgtttagtttctttctttcttcttctccttttcttttcttttttctttggttttttgtttgtttgtgtgtttgtttgttttgttttttgtttgtttgtttgtttgtttttttgagacagggtttctctgtatagccctggctgtcctggaactcactctgtagaccaggctggccttgaactcagaaatccatctgcctctgcctcccaagtgctgggattaaaggcgcgcgccaccacgcccggcttttgtttggtttcttaatctccattcacagatgaaagaagaaaggcacctggggtctcagttacctatatcaggatcactaacaatgagtaagacgcagtctagcccatgtgtccaggcctacccaccaccccagcctgcctttctttacagatagtcaccttcaaaaatcacacaatagaggcacaatcacaaagggcatttttttcctttaacatttatttatccatttaatgtatatgaatacactattgctctcttcagacacatcagatcgcattacagatggttgtggaccaccatgtggttgctgggaattgaactcaggactgctgggtagtggtggtgcatgcctttaatcccagcacttgggaggtagaggcaggcagatttctgagttcgaggccagcctggtctacagagtgagttccaggacagccaggactaaacagagaaattctgtcttgaaaaaacaaaaaacaaaaaaaacctcaggacttctggaagaacagtcagtgcaactaacccagcccacacagagggctctgaccaacagatctgaacctgacaaagattgctgtggccttgggggttcttatcactatgactgtggttttcgctacccagtccctctgtagtggggaagtggagctggctaggagggatagactattcctaactgcattctgggaggggattggatgcaaaggttcacacagtggggagtattcacatcacaggaaggatgtttacacggtggggagcatttataccacagggcattcacaccatggggcacactcacaggataggaaatgttcatatcccggggagtgttcacacctgggggtggaaggtgttcacaccttagagagtgttcacactgtagaaagtgacaaagtcgaaagctgctttgctctgctgagcccatggataaccatttatgggcacaaggttgtctttgtctctcactatagtacatctcacacagcccccaggtcctgatgggagggtaaacagacatgggagggtaaacagacataagagggctatgaggctgggaatccaaaggtcttgacctggcgaaagagtcctccagggcccaccctctaccaattcaggtctggagagctgtggacacatcgagatttcaccccctgttgtccgcctgggggaccctgtcctggcctcttgcaccatcagcccaaactgcagcaaactggaccaacaggcaaagatcttatggagactgcaagatgagcccatccaacctggggacagacagcatcatctgcctgatgggacccaagagtccctcatcactctgcctcacttgaactacacccaggccttcctcttctgcttagtgccatgggaagacagcgtccaactcctggatcaagctgagcttcacgcaggctgtaagtccctccagccatctacccatctgcttccaatgcccctctgccaaaaccagggagagctaagacctcgctcaagtagccctttgtgagtacgacagaaggtgtggttctttctatcattctataattctctaataaagaagctgacatctggcaagggcaagtgacctattgaaggccatacccacaggggttcttgtagagccaaccacctgtctatttggctgtttagcaagctcaggttcttggccataagaggggcttacttccagctcctcctcagtcgggtcccagctttctttccaaattgagcaggatggagtctgtgccaagctgagatataaagaacaaataataaccaaggcatgataccacctctctactccgagctgaggtttgcaagccgggtttctctaacaaccctggctggtcttgattcagacttctgtctgcctctgcctctcgaatgttagaattaaaggtgtgcaggtgtgcaccaccaccgactgtcaaatgcacacccccatcctgccgcccaggatctctatgatctttgagagttccagcgcagctaggactacatagtaagaccttgtctaccccattccctcaaaaagaaatgggtgccagggttgaggatgtagccctgtagtaaaacacatactcatcaagagcaaggttctgggttctaatccacactaagcaatgagagagccaggcatggagtcacacttctgtggtcttggtgctacttggaaactgagacaggaggatggtgaattaggaagtagcacagacggtatcacgagtcctgtctccagcagtgatggggaagctgccacctgcgtgaacacagttgggagctgcctatagagaggaagtcacttagcccctgtatgtgctgcttttctgttgctatgacacaacaccaggactaggaaaacttataaaaagacagcctttaattggccttatgttccagacagttcacaacggtggagcaaaagctcggtgacagaagcagctgagagtttacatcttgaagagcaagcaggagacagaggactaattggagataggacaaatcttttggaacctcaaagctcaccctcagtggcacaatacctcctccaacaaggcttccaaaacagttccgctatctgggaactaagtattcaaacatgagcctttgggggtccattctcaatgaaaccaccacagaagtctaggagagccatgtggtatcacacatctttaatcccagcactcaggaggcagaggcatgtggatctcttagtttgaggctagcaggctggtcttcagagatgagtttcagattagtcaggaccacagagaaacactgtctgggaagaaaaagaaggaggaggaggaggaggaggaggaggaggaggaggagggaaaaacctaggagagagaaatttattagcattacctcctctttacagataaagaaactgaggcagagagcagttcagtcacttaaggataaaatggctaatgaatgactgactaaaccataataaaactcaggctgtactgtcaccgacaaaggggccaccagggtgctaagggtctgggatgtctgctcctcacaggtccacactacagaaggaacagtccaccaaggaagtaaggccacaagtacacacacacacacacacactcacacacaccccgagagggctcctaacattcttttcaccctatccagatccccctgccagcccctcaaacctatcctgcctcatgcacctcaccaccaacagcctggtctgccagtgggagccaggtcctgagacccacctgcccaccagcttcatcctaaagagcttcaggtatgtaggatctccatggcagccccttcctccaggtcccggtttgggacacaagtccctataggggtgaggagatatgatgaggtgtggggtggggctggggagggtggagggcagagaaagagagagaagatagagaagatccttgccttcttcctctgcttggcaccaaagcccagcctgttggcaggagccgcgccgactgtcagtaccaaggggacaccatcccggattgtgtggcaaagaagaggcagaacaactgctccatcccccgaaaaaacttgctcctgtaccagtatatggccatctgggtgcaagcagagaatatgctagggtccagcgagtccccaaagctgtgcctcgaccccatggatgttggtgagtgacactgggtatgtgaaaatggagaagtccccaaattagaagacccagaggtacataaagaggaaatacagacctaggcacagacagagagattttggaagacctggagagaggcagaaaagagagaaatgaggaccagaggctatggacatgttcgttcttttatcttttttttttccttttttctttttggtttttcgagacagggtttctcttttagctctggctgtcctggagctcactttgtacaccaggctggcctcgaactcagaaatccgcctgcctctgcttcccgagtgctgggattaaaggcatgcgccaccatgcccggctgtcttttatcttatttattcattggcttttttaaagatttatttattcatttacattatttatttatttatttatttatttatttatttatttatttattcatgtacatgagtacactgtccctgtcttcagacacaccagaagagggcatcagatcctgttacagatgtttgtgagccaccatgtggttgttgggaattgaactcagggcctctggaagagcaagcagccagtgctcttaacctctgagccatctctctagcatgagttgctgggaattgaactcaagacctctggaagagcaatttgtgctcttaaccactgagccatctctctagccctattcattggtttttcaagacaaggtttctctgtgtagccctggctgtcctggaaattgctgtgtagacctggctgacttcaaaacgtgtcaccaccacctgcctcatcttatttatttatttatttacttacttatagggtcaatgcacacatatatacacatatggaggccagaggatctttctggagccattctctcccctgccttgaaggcagtgtctctcttgtctctgatgctgcccttggctccaggcaatatgacctggaagcctcagagtgcttttcctgtctccacctcccagtttgttgcaatactgatggtattacagatagacacaattatattgggctttaaaaaaaagatttatttattttatttatgtgagtacactgtagctgtcttcagacacaccagaagagggcatcagatcccattacagatggttgtgagccaccatgtggttggtgggaattgaactcaggacctctggaagagcaaacagccagtgctcttaaccactaagccatctctccagttttttcttttttaaaatgtacattagtgttttgcctgcatgtatgtctgagtaagagtgtctgatcccctggatcaggagttacagacggctgtgaactgccatgtggttgctgggaattgaacctaggtcctccggaagagcagtgttcttaaccactgagtcatctctccaaccctgcattgggctttttggtgctgtcaggcttgcatcactagctagctctttttacccaatgatccatcaccccaggtttcagcttattccttaacgtgcccccacctcatgcaaagctgtggaggtcctaaagatagacagggcattggaataagcctcaaaggccccaccctcggaatattaaaacaatttaggtggcaaaataaataaaatacagtatcgggtaattttaagacattgacagctaactagacggttgggggagctgagggagcaagatatccctggatatctggaaagaaaacaatgtaagcaaatgtaacaaccagttagaggtaacaacctagtaagaaatactgacactggtacccaagcacagctagagatcatggcagcagagaaatggagactgaaggaaaggggagctaagccagagccctctccatcggaaagtttgacaaccccacctcctgcagtgaaattggagcctcccatgctgcaggccctggacattggccctgatgtagtctctcaccagcctggctgcctgtggctgagctggaagccatggaagcccagtgagtacatggaacaggagtgtgaacttcgctaccagccacagctcaaaggagccaactggactctggtgaggccgagaacaacctagagatggaggtgggggatggagagagggctagttggatttagtgtcacctcccacacaccaggtgttccacctgccttccagcaaggaccagtttgagctctgcgggctccatcaggccccagtctacaccctacagatgcgatgcattcgctcatctctgcctggattctggagcccctggagccccggcctgcagctgaggcctaccatgaagggtgagaagccaggagaagccttcagagctcagttcaggacccaacccctctgccctccatcaaaaccctctcatcttggggctggagagatagctcattggttaagagcactgactgctcttctagaggtcctgagttcaagtcccagcaaccacatgatggctcacaaccatctgtaatgggatccgatgacctcttctggtgtgtctgaagacagctacagtgtattcatagaaatttaaaacaaaaaaaaaaaaaggctcaagaaagtaaatgtcctaatttttaaaaagatttattcaggggctggtgagatggctcagcgattaagagcactgactgatcttccagaggtcctgagttcaattcccagcaaccacatggtggctcaaaaccatctataatgggatctgaaatggtgtgtctaaagacagctacagtgtactcatatacataaaataagtaaatctttgggaaaaaaagatttatttatttattttgtgtatatgacacactaaaagagggcatcagatcacattgtagatggttgtgagctaccatgtggctgctgggaattgaactcaggacctctggaagatcagtcagtgctcttaaccattgagccatctttccagccccaaatagtcatactttaaaaaaaaaaaacccacaaaaccctctcatcctgtctatccatctacatcctcccacatccatctacagcccccaccatcagactggacacgtggtgtcagaagaagcaactagatccagggacagtgagtgtgcagctgttctggaaggtgactctctgaaaccctctccaaccctcctaacagagtccccaatatagtgctcaaaaactgcagtgtgcctgggaggcaatttgcaagccctttacacataccacagaagctgggtagtggccttggggagagactgcaatgcagggttctggggtcacctgtaccccaaagggtccacttagagaatagttccgcaagtgtcacgtgtgctgtctggcttcttccttctttctctcctagttcttgccacaggggaagagggggaggggaggaaggacttagggcccagttcttatggctggtccatgcctctcaggtactgactaattcacaccacagtgaactagacaaccccctcaccgtgttcttcctcacccaccgcagccaacgcccctgcaggaagacagtggacagatccagggctacctgctgtcctggagttccccagatcatcaagggcaggacatacacctttgcaacaccacgcagctcagctgtatcttcctcctgccctcagaggcccagaacgtgacccttgtggcctacaacaaagcagggacctcttcacctactacagtggttttcctggagaacgaaggtaaagggggctggcagctgagcagcagagagcagtgtgggaattttgaggttggactgactatgtgcctacctgtctagtcaaccacttgttaagagagtggcctggacaggtgactttctttcctggcccctgtcacctgcaggtgtatgcactgacattgcctctgagggcagtaaactttgagccaactttgttttgttttggtttgttttgtttgttttgttttgttttgttttcgagacagggtttctctgaatagccctggctgtcctggaactcactctgtagaccaggctggcctcgaactcagaaatccgcctgaatctgcctcccaagtgctgggattaaaggcgtgtgccaccatgcccggcatttgagccaacttttaaattattattcttgctagccagaactaggttaatctgggagaatatacatacctgcatatacatgttgtacatatggatggatggatggatggatggatggatggatggatggatggatgataaagtatgattcccgcttacaagttgtatgtataaatatagcagctggcagacaacctcaaatgtcattcttagggtgctgtgcactttttttggagacaggatttcccatcagtctgaaattcactgattagaatctccgtcagggttctacctgcctctaccttccctgtgctggggttataaatgccacatgcctgtttcctttgctgttgtttccatatggaaactggggaccaaattcactgcttgccttataagcactttaccaattaaatgatctctccagccctgagctttgagctttgtttaaaatttgatcatgtattttatgtatataagtgccctgtcttcttgtaagaaggaggaatcagatcccattacagatggttgtgaaccaccatgtggttgctgggacttgaactcaggacctctggaagagcagccagtgttcttaacctctgagccatctctccagcccctgagctgtgtgatcttaagtaagcctctcttgtttcccattttttactcattgataaaatggagacaactagtcaggcgtggtggtgcacgcctttaatctcagcactcgggaggcagaggcaggtggatttctgagttcgaggccagcctggtctacaaagtgagttccaggacagccagggctacacagagaaaccctgtctcaaaaaaaccaaaaaaaaaaaaaaaaaaaaaaaaggagacaactatagaagctccctggtatgactgttgaagaactcggtgaatcacatatattaagctaaatggtgccaggctctgtgctaggcttgttctgcgcaccttcctttaacacacaagcctctacaaagcgggaatttttttgttgtcactttccctttacagatgtggagcttggtgatcaggtattgacataccctggatcacaggtctgttggcagcaaaggcaaggtttggatccaagtgtctgctactgaggcctgcgtacttttcgtcttcactcctattccctgctttacctccaggtccagctgtgaccggactccatgccatggcccaagaccttaacaccatctgggtagactgggaagcccccagccttctgcctcagggctatctcattgagtgggaaatgagttctcccagctacaataacagctataagtcctggatgatagaacctaacgggaacatcactggaattctgttaaagggtgaggtgggcctggggcaaaggaatgggctgagggataagaagaaggaacagagggaggggtgcatgtctagaggtagcttggaacctccctatagaggcagcctccccagccttttctgaaaccttacctggggaaagttcttcctcccctctagttctctgttccacgttccctgtgtgacttccatcaaatgcgctaaaagagatctctgagcttagccccaaggtcaaaatcaggccttgcagaaatgggagtctgaggctgggtagcagaggttagctcccacccttagtgctgtcccattttctctctgcagacaacataaatccctttcagctctacagaattacagtggctcccctgtacccaggcatcgtgggacctcctgtaaatgtctacaccttcgctggagagagaggtttgtctacccacagtgttcccaaaatcctctcctctctccctatctgggctctagcaatggggagtatgggaataaacacactcttttacttctggcctctgagtcgggtgttttccatcatggctcacagtggactccccaaagctgggcagaaggtggggtagaagacagggagctgtgaactggagaaaatcggggttggagtcagtttcacagaatcaatccatagccccaacagaaatccagggtcacatctgaaagaattgaaccaagtattcagagggtgagtggctgaaaccagacaccaagtcggataaaaccagatgtggcaaaaatcagacagcagctagaactggattcaaacccaggctctgcctctgggagccataaactgaattcacatgacatcctggtggggtctacctctgaccctagcaactctgatgaggtagcattgtgatttggggaacagcctgagccatgtgagattcgcccccccccaaacagagtaccctcttagaagggatatctatctatctatctatctatctatctatctatctatctatctatctatctatctatctatctatctatctatcgatacctatctcttccccactcaccccccatttgcttttggtttggggttttgtgtttgatttttgttggttttgccgttgctttaattcaattattattatgtgtgtgtgtgatgtgtgtgaatggacacacacatgccagagtgcctgtggaggtcagaggacagctctgtacactcagttctctcagtccacctttgtgtggtgtgctagttttcattatcagtgtgacagaacctcgagtcacctggtctagggaacctcgtttgagcaattgcccacatcatatttattggcctgtgattacttttatgagaaatcatcataattgattgatagctgatgtgggagggcccaacccactacaggaagtgccacctccacttaggaggcagatatggctagatgagcgagtcaaagagctggtcagtgttagcagcattcctcctccgtgggttccacttccatttctccttgaatgtactctctgacctccctcaacaaggagttaagactttggtcctggtctaatcacagcaacagagaagcaaagagcatggttttagaccatagcccgggctggcctcaagtacacagcaatcctcctgcctcaatcttcagcgtgctaggattaaagacatgtacaagcacactcatctccttgagttcttacctctcgtccatctagagaatgtcccagatcctgagtccagtcaggctcacttgccctgattatatcagccctttcacctcctctctctctctccacagctcctcctcatgctccagcgctgcatctaaagcatgttggcacaacctgggcacagctggagtgggtacctgaggcccctaggctggggatgatacccctcacccactacaccatcttctgggccgatgctggggaccactccttctgtgagtcgatccttagctccccacaagcccaggaatcctagaaggggtgttcctcggcacatacagaggtgtgttagcatcccaagctgaccatatgctccacccacagccgtcaccctgaacatctccctccatgactttgtcctgaagcacctggagcccgccagtttgtatcatgtctacctcatggccaccagtcgggcagggtccaccaacagtacaggccttaccctgaggaccctaggtaagaggccgggacagtgttcgctgttgggagggtgccccactttgtctctcaaaaagtcccgactttaagctgggcagtggtggcagagacaggcgaagttctgagttcgaggccagcctggtctacagagtgagttccaggacagccaggactgattttgccaggtgtggtggcacacatctttaatctcaacactgaggacacagaggcaggtagagctctgtgagtatacagttgttcggatctacatagtttcaggccaaccagggctctctcaaggcgataagtaaatattccaggacagctagggctatacagagaaactctgtctcgaaaaaccaaaaaagagcaagaagaagaagaagaagaagaagaagaagaagaagaagaagaagaagaagaagaagaagaagaaaagtaaataaaaagaaatcccaatttttaaagagaggagagattatatatatatatatatatatatatgtttgtttgttgatgttgttgttgttgttgttaatttaaaaagttaaaaatcatgcagggcagcagtgacgcatgcctctgatcccaggcctcaggaggcagaggcccgaagatctctgagttcaaggccagcctggtctacagagtgagctccaggacagccagggttacacagagaaaccctgtctcaaagaaaacaaaaaaagaagtcttaattttgagaacaataggaagctacctttggacctgctaatctgagaggagaccagggcctgttcaagaacactcttctgtgagaggagacccagccctacccacctgacttacacacactactgcccagggctctttaacccttttaaaatacatatatttatttatttcatgtatgtgagtacactgtcactgtcttcaggcacactagaaggtagcatcggatgcccattacagatggttgtgagccaccatgtggttgctgggaattgaactgatgacctctggaagagcagccagtgttcctcaccactgagctctctctcccgccctaacctctccactttttttgttgttgttttttccagacagggtttctctgtatagccctggctgtcctgaaactcacttttagaccaggctggcctcgaactcagaaatctgcctgcctcccgagtgctgggattaaaggtgtgcgccaccacgcctggccagtcccttttttttttacacaagaaatttttacataattctgggcatgtatgcatgtaaaacataaccagatcaaacacttaactgataacaaaccatgcatttattttgaaacgattccttgatcagcatataaattatctttattatagactaagcaagcccacatactaatcacatggatgttcttgcttctttttacccagataattaactgttggctaaatgttggatactgcagggcaaagagcatcttagccaccttcagcatttttcagagctaaccaattttttgatctttgcagtcatcaatgctgaggacacattgcataaaaaagtaatcattttaacatgattcaatcagaagatacactaattcaatgtctgcatgctgaggattgatggcaggaaaatgttaagtctttggtttagcgggaggtagtagcgcacgcctttaatcccagcactcagggggcagaggcaggcggatccagtcaacctggtctataaactgagtttcaggacagccagggctacacagagaaaccctgtctggaaaagccaaaccaaaccaaacaaaaacaaaacaatagtcttagctttgctttccatgattaaaacatacgttcctgcaatggcaagaccctctgaatttacagtaaacacactgagattacagtagtcttgaatctgagccaaggtgtttcgggcagtgcttggtgatgttgtgtgacgtgatggtgtatgcacagtgcaagcaaagtgtgtgtgtgcaaaccaagtgcacacggattagaaccaaggctgcagtgaacttgtgtgatgtaacacaggtgaagtatgttggaagattcattatgtgtatgtgttggggtttttaaaaaattatctaatatttatatttcatgtgttttgcctgtatgtatgtctgtgtgagggtgttagatcctctggagccagagtcacagacaggtgtgagctgtcatgtgggtgctgggaattgaacccgggtcctctggaagagcagccagtgctcttaaccactgagccatctctccagcctccaaaccttccattcccccccacccctatggttttaaagacagggtatctctgtgtaacagttctagctgccctggaactcactctgtagacaaggctggcctcgaactcacagaaatctacctgcttctgcctcccaagtgcaagtatgtgccacgactgcttggctgttttgttttgtttttaattaccttttagatgttattcttgtttttttgttttgttttgttttttgttttttcgaggcagggtttctctgtatagccctggctgtcctggaactcactctgtagaccaggctggcctcgaactcagaaatccgcctgcctctgcctcctgagtgctgggactaaaggcgtgcgccaccacgcccggctttagatgttattctttaggaacctttcaacctgccaacatttgactctctccacattcagcaccactgagttcatgacccacagtggaaaagccacaccctaaactcttcttgctttctgtctctcaccccagatccatctgacttaaacattttcctgggcatactttgcttagtactcttgtccactacctgtgtagtgacctggctctgctgcaaacgcaggtgagtggcttccttttacccatgggtgcggaagtcccttcctgccttcccagacttccgggccccaatctgggaggtctgtcctaacatctcttcccctcttcagctgccagatggcaagctgacccaaacttcacttgtctccttctgcagaggaaagacttccttctggtcagatgtgccagacccagcccacagtagcctgagctcctggttgcccaccatcatgacagaggtaatcatgaggcagagaggtgtataaactgtgactggcagacaaggcagcgtcattaaaggaacacacacctgagccccacttccaaccagacacacacacacattctgctttggagagatgtaggcctgagtttgactctccaagattggtcacctcactacacaatggatgcgtgggtggcagagggtgggttgggctgggggtcatgtgtcagggacatggtaggaatggacagctgccaggcaagtatgtccctttgtgctctgccacatagcaacaagggagatgccataactacctcatctctggaaggaacgatgtgtggagcagacatgtgagacaaaccatgccgtattgtgtatatccctgtgttcaggaaaccttccagttacccagcttctgggactccagcgtgccatcaatcaccaagatcactgaactggaggaagacaagaaaccgacccactgggattccgaaagctctgggaatggtagccttccagccctggttcaggcctatgtgctccaaggagatccaagagaaatttccaaccagtcccagcctccctctcgcactggtgaccaggtcctctatggtcaggtgcttgagagccccaccagcccaggagtaatgcagtacattcgctctgactccactcagcccctcttggggggccccacccctagccctaaatcttatgaaaacatctggttccattcaagaccccaggagacctttgtgccccaacctccaaaccaggaagatgactgtgtctttgggcctccatttgattttcccctctttcaggggctccaggtccatggagttgaagaacaagggggtttctagaactttgggggtccttgtatcttgaagaccctgccctattcagaggagaagagccctccgctgaaatctactggccctgagagaagcagaaaggcccagtgtgtctctgtctctggcccctagcacctctcctctactctgagcttctcaggctataccctgaggtcacccactctcacactctaaggttcagatagatactgcttacagcccaatggtcaccattcgtctttcatataatttcagtccattgaactgattgtaggttttgagttggggctggtattttcagaaattctggctggacgtggtggtacatgcctagcatcccaacatctgggaggaagatgcaggaagattgcaagttccaggccagcctgggctagcctacatagtgagatccaatctcaaaaattatgctgggtgtggtggtgcatgcctttaatcccagcactcgggaggcagaggcaggtagatttctgagttcgaggccagcctggtctacaaagtgagttccaggacagccagggctatacagagaaaccctgtcttgaaaaaaaaaattaagcaaaagctgaataaataaagttttttttatgacatgtacttgttttgtggggagtggggattcagaggcagaggtcagaagacacctaccttgtgggaattaactctggtctccagcatgtggatcttgagaagtggactcaaagcttagtgacaagcaccgcgttacccatggaggcatcttattggtcccagaaaagaatctcttgagcatagcttaagtgtcttctacccttgtttgttttttgtctctgcttgcttgtttttctttttatgtattataaataagtacaatgttgctgtcttcagacacaccagaagagggcatcagatctcaatactggtggttgtgaaccaccatgtggttgctgggatttgaatttaggacctttggaagagcagtcagtgctcctacccgctgagccatctcttcagtccagtttatttgtttttcaagacagggtttctctgtgtaacagcccaacctatcctggaacttactctatagatcaggctggcctcaagatccacctgcctctgccttaaatgctgggaataaaggtgtgcaccaccaccaggaagtggctttcactttcagggcccaacagtcaagaaggtatttctcagaatcattt